European Patent Application EP 4 252 542 A2, published October 4, 2023. Title: LIVESTOCK FEED ADDITIVE. Applicant: Delacon Biotechnik GmbH. The sequence listing filed with the application follows.

SEQUENCE LISTING (4 sequences)

SEQ ID NO: 1 - DNA, 22 bp, synthetic construct
  misc_feature 1..22: note = Primer
  source 1..22: mol_type = other DNA
gcgggaaatcgtgcgtgacatt

SEQ ID NO: 2 - DNA, 24 bp, synthetic construct
  misc_feature 1..24: note = Primer
  source 1..24: mol_type = other DNA
gatggagttgaaggtagtttcgtg

SEQ ID NO: 3 - DNA, 25 bp, synthetic construct
  misc_feature 1..25: note = Primer
  source 1..25: mol_type = other DNA
ctagcctgaggagctgctgcgacag

SEQ ID NO: 4 - DNA, 26 bp, synthetic construct
  misc_feature 1..26: note = Primer
  source 1..26: mol_type = other DNA
gttccctgctctctgtcggctcggct